European Patent Specification EP 4 557 954 B1, published May 20, 2026. Title: The control of nematodes. Applicant: Magrix (Pty) Ltd. Application IB. The sequence listing filed with the application follows.

SEQUENCE LISTING (2 sequences)

SEQ ID NO: 1 - protein, 251 aa, Jatropha curcas
AGSTPTLTITYDAAADKKNYAQFIKDLREAFGFSYSSHEIPVLRATVAPNQKFIVAKVINVANLEVSLGLNVVNAYLVGYKVGGTSYFFNDPESLADAKTYLFTDTKQQTLSFTGSYADFLSRANVHREDVDLGVQALDNYIYTLEKSSKPADIAKPLVGFIEMVPEAARFKYIEKKVLSQISKTLRPGGDIISLENNWGDLSYQIQKCVNGVFLKPVQLQRENYTNILVNNVTQVAGVMGVLLNAVNYKV

SEQ ID NO: 2 - DNA, 756 bp, Jatropha curcas
  source 1..756: mol_type = genomic DNA
gctggtagtaccccgaccctgaccattacctatgatgccgccgcagataaaaagaattatgcacagtttatcaaggacctgcgtgaagcctttggttttagttatagtagtcatgaaatcccggtgctgcgcgccaccgtggcacctaatcagaaattcattgtggcaaaagtgattaatgtggcaaatctggaagttagtctgggcctgaatgttgtgaatgcctatctggtgggctataaagtgggcggtaccagttatttctttaatgatccggaaagtctggccgatgccaaaacctatctgtttaccgataccaaacagcagaccctgagttttaccggcagctatgccgattttctgagtcgtgcaaatgtgcatcgtgaagatgtggatctgggcgttcaggccctggataattatatctataccctggaaaaaagcagtaaaccggccgatattgcaaaaccgctggtgggttttattgaaatggtgccggaagcagcccgctttaaatatattgaaaagaaagtgctgagccagattagcaaaaccctgcgtccgggtggcgatattattagtctggaaaataattggggtgacctgagctatcagattcagaaatgcgtgaatggtgtgtttctgaaaccggtgcagctgcagcgtgaaaattataccaatattctggtgaataacgtgacccaggtggccggcgtgatgggcgttctgctgaatgccgttaattataaagtgtaa